European Patent Application EP 4 756 029 A1, published June 10, 2026. Title: TOLL-LIKE RECEPTOR AGONISTS AND USE THEREOF. Applicant: HAICHANG BIOTECH CO., LTD. Application CN PCT/CN2024/111218, filed August 9, 2024. The sequence listing filed with the application follows.

SEQUENCE LISTING (4 sequences)

SEQ ID NO: 1 - DNA, 26 bp, synthetic construct
  source 1..26: mol_type = other DNA
  unsure 1..26: note = all phosphodiester bonds are phosphorothioated
tcgaacgttcgaacgttcgaacgtat

SEQ ID NO: 2 - DNA, 22 bp, synthetic construct
  source 1..22: mol_type = other DNA
  unsure 1..22: note = all phosphodiester bonds are phosphorothioated
tcgaacgttcgaacgttcgaat

SEQ ID NO: 3 - DNA, 34 bp, synthetic construct
  source 1..34: mol_type = other DNA
  unsure 1..34: note = all phosphodiester bonds are phosphorothioated
tcgaacgttcgaacgttcgaacgttcgaacgtat

SEQ ID NO: 4 - DNA, 38 bp, synthetic construct
  source 1..38: mol_type = other DNA
  unsure 1..38: note = all phosphodiester bonds are phosphorothioated
tcgaacgttcgaacgttcgaacgttcgaacgttcgaat